European Patent Application EP 4 692 313 A1, published February 11, 2026. Title: L-glutamic acid-producing bacterium and method for producing L-glutamic acid. Applicant: Ajinomoto Co., Inc. Application WO PCT/JP2023/047152, filed December 28, 2023. The sequence listing filed with the application follows.

SEQUENCE LISTING (10 sequences)

SEQ ID NO: 1 - DNA, 1542 bp, Corynebacterium glutamicum
  source 1..1542: mol_type = genomic DNA
ttgaaaaagtccgattacctgaggaggtattcaatgtctgatcgcattgcttcagaaaagctgcgctccaagctcatgtccgccgacgaggcggcacagtttgttaaccacggtgacaaggttggtttctctggcttcaccggcgctggctacccaaaggcactgcctacggcaatcgctaaccgggctaaagaagcacacggtgcaggcaacgactacgcaatcgacctgttcactggcgcatcgaccgcccctgactgcgatggcgtacttgcagaagctgacgctatccgctggcgcatgccatacgcatctgatccaatcatgcgtaacaagatcaactccggctccatgggatactccgatatccacctgtcccactccggccagcaggttgaagagggcttcttcggccagctcaacgtagctgtcattgaagtcacccgcatcactgaagacggacacctcatcccttcttcctccgtgggtaacaacgttgagtggctcaacgctgcagagaaggtcatcctcgaggttaactcttggcagtccgagaacctcgagggcatgcacgacatctggtctgtaccagcactgccaaaccgcatcgctgtgccaatcaacaaggccggcgaccgcatcggtaagacctacatcgaattcgacaccgacaaggttgtcgcaattgttgaaaccaacaccccagaccgcaacgcaccatttaagcctgtcgatgacatctctaagaagatcgccggtaacttcctcgacttcctcgaaggtgaagttgcagctggccgtctttcctacgatggttacgtcatgcagtccggcgtgggcaacgtgcctaatgctgtgatggcaggcctgctggagtccaagtttgagaacatccaggcttacaccgaggttatccaggacggcatggttgaccttatcgacgccggcaagatgaccgttgcttctgcaacctccttctccttgtctcctgagtacgcagagaagatgaacaacgacgcaaagcgttaccgtgagtccatcatcctgcgcccacagcagatctctaaccacccagaggtgatccgtcgcgtcggcctgatcgccaccaacggtcttatcgaagctgacatctatggcaacgttaactccaccaacgtttctggctcccgcgtcatgaacggcatcggcggctccggcgacttcacccgtaacggctacatctccagcttcatcaccccttcagaggcaaagggcggcgcaatctctgcgatcgttcctttcgcatcccacatcgaccacaccgagcacgatgtcatggttgttatctctgagtacggttacgcagaccttcgtggcctggctccacgtgagcgcgttgccaagatgatcggcctggcacaccctgattaccgcccactgctcgaggagtactacgctcgcgcaacctccggtgacaacaagtacatgcagacccctcatgatcttgcaaccgcgtttgatttccacatcaacctggctaagaacggctccatgaaggcataa

SEQ ID NO: 2 - protein, 513 aa, Corynebacterium glutamicum
LKKSDYLRRYSMSDRIASEKLRSKLMSADEAAQFVNHGDKVGFSGFTGAGYPKALPTAIANRAKEAHGAGNDYAIDLFTGASTAPDCDGVLAEADAIRWRMPYASDPIMRNKINSGSMGYSDIHLSHSGQQVEEGFFGQLNVAVIEVTRITEDGHLIPSSSVGNNVEWLNAAEKVILEVNSWQSENLEGMHDIWSVPALPNRIAVPINKAGDRIGKTYIEFDTDKVVAIVETNTPDRNAPFKPVDDISKKIAGNFLDFLEGEVAAGRLSYDGYVMQSGVGNVPNAVMAGLLESKFENIQAYTEVIQDGMVDLIDAGKMTVASATSFSLSPEYAEKMNNDAKRYRESIILRPQQISNHPEVIRRVGLIATNGLIEADIYGNVNSTNVSGSRVMNGIGGSGDFTRNGYISSFITPSEAKGGAISAIVPFASHIDHTEHDVMVVISEYGYADLRGLAPRERVAKMIGLAHPDYRPLLEEYYARATSGDNKYMQTPHDLATAFDFHINLAKNGSMKA

SEQ ID NO: 3 - DNA, 1542 bp, Corynebacterium glutamicum
  source 1..1542: mol_type = genomic DNA
ttgaaaaagtccgattacctgaggaggtattcaatgtctgatcgcattgcttcagaaaagctgcgctccaagctcatgtccgccgacgaggcggcacagtttgttaaccacggtgacaaggttggtttctctggcttcaccggcgctggctacccaaaggcactgcctacggcaatcgctaaccgggctaaagaagcacacggtgcaggcaacgactacgcaatcgacctgttcactggcgcatcgaccgcccctgactgcgatggcgtacttgcagaagctgacgctatccgctggcgcatgccatacgcatctgatccaatcatgcgtaacaagatcaactccggctccatgggatactccgatatccacctgtcccactccggccagcaggttgaagagggcttcttcggccagctcaacgtagctgtcattgaagtcacccgcatcactgaagacggacacctcatcccttcttcctccgtgggtaacaacgttgagtggctcaacgctgcagagaaggtcatcctcgaggttaactcttggcagtccgagaacctcgagggcatgcacgacatctggtctgtaccagcactgccaaaccgcatcgctgtgccaatcaacaaggccggcgaccgcatcggtaagacctacatcgaattcgacaccgacaaggttgtcgcaattgttgaaaccaacaccccagaccgcaacgcaccatttaagcctgtcgatgacatctctaagaagatcgccggtaacttcctcgacttcctcgaaggtgaagttgcagctggccgtctttcctacgatggttacgtcatgcagtccggcgtgggcaacgtgcctaatgctgtgatggcaggcctgctggagtccaagtttgagaacatccaggcttacaccgaggttatccaggacggcatggttgaccttatcgacgccggcaagatgaccgttgcttctgcaacctccttctccttgtctcctgagtacgcagagaagatgaacaacgacgcaaagcgttaccgtgagtccatcatcctgcgcccacagcagatctctaaccacccagaggtgatccgtcgcgtcggcctgatcgccaccaacggtcttatcgaagctgacatctatggcaacgttaactgcaccaacgtttctggctcccgcgtcatgaacggcatcggcggctccggcgacttcacccgtaacggctacatctccagcttcatcaccccttcagaggcaaagggcggcgcaatctctgcgatcgttcctttcgcatcccacatcgaccacaccgagcacgatgtcatggttgttatctctgagtacggttacgcagaccttcgtggcctggctccacgtgagcgcgttgccaagatgatcggcctggcacaccctgattaccgcccactgctcgaggagtactacgctcgcgcaacctccggtgacaacaagtacatgcagacccctcatgatcttgcaaccgcgtttgatttccacatcaacctggctaagaacggctccatgaaggcataa

SEQ ID NO: 4 - protein, 513 aa, Corynebacterium glutamicum
LKKSDYLRRYSMSDRIASEKLRSKLMSADEAAQFVNHGDKVGFSGFTGAGYPKALPTAIANRAKEAHGAGNDYAIDLFTGASTAPDCDGVLAEADAIRWRMPYASDPIMRNKINSGSMGYSDIHLSHSGQQVEEGFFGQLNVAVIEVTRITEDGHLIPSSSVGNNVEWLNAAEKVILEVNSWQSENLEGMHDIWSVPALPNRIAVPINKAGDRIGKTYIEFDTDKVVAIVETNTPDRNAPFKPVDDISKKIAGNFLDFLEGEVAAGRLSYDGYVMQSGVGNVPNAVMAGLLESKFENIQAYTEVIQDGMVDLIDAGKMTVASATSFSLSPEYAEKMNNDAKRYRESIILRPQQISNHPEVIRRVGLIATNGLIEADIYGNVNCTNVSGSRVMNGIGGSGDFTRNGYISSFITPSEAKGGAISAIVPFASHIDHTEHDVMVVISEYGYADLRGLAPRERVAKMIGLAHPDYRPLLEEYYARATSGDNKYMQTPHDLATAFDFHINLAKNGSMKA

SEQ ID NO: 5 - DNA, 37 bp, Corynebacterium glutamicum
  source 1..37: mol_type = other DNA
ccaagcttgcatgccatgcttgtgggcgtacctgtcc

SEQ ID NO: 6 - DNA, 37 bp, Corynebacterium glutamicum
  source 1..37: mol_type = other DNA
cggtacccggggatcttagacgatggtccagtcttcc

SEQ ID NO: 7 - DNA, 1602 bp, Corynebacterium glutamicum
  source 1..1602: mol_type = genomic DNA
atgattttaggcgtacccattcaatatttgctctattcattgtggaattggattgtcgataccggttttgatgtagcaattatcctggtcttggcgtttttgattccacgtatcggccgactggccatgcgtattatcaagcagcgagtggagtctgcagccgatgcggacaccactaagaaccagctcgcgttcgctggcgttggcgtttatatcgcgcaaattgtggcgtttttcatgcttgccgtctccgcgatgcaggcttttggtttctctctcgcgggcgctgcgattccggcaaccattgcgtcagctgccattggtcttggtgcgcagtcgattgttgcggacttcttggccggatttttcatcctgacggaaaagcaattcggcgtgggtgactgggtgcgctttgagggcaacggcatcgttgttgaaggcaccgtcattgagatcaccatgcgcgcgaccaaaattcgcacgattgcacaagagaccgtgatcatcccgaactccacggcgaaagtgtgcatcaacaattctaataactggtcgcgtgcggttgtcgttattccgatccccatgttgggttctgaaaacatcacagatgtcatcgcgcgctctgaagctgcgactcgtcgcgcacttggccaggagaaaatcgcaccggaaatcctcggtgaactcgatgtgcacccagccacggaagtcacaccgccaacggtggtcggcatgccgtggatggtcaccatgcgtttcctcgtgcaagtcaccgccggcaatcaatggctggtcgaacgcgccatccgcacagaaatcatcaacgaattctgggaagaatacggcagcgcaaccactacatcgggaaccctcattgattccttacacgttgagcatgaagagccaaagacctcgcttatcgacgcctccccccaggctcttaaggaaccgaagccggaggctgcggcgacggttgcatcgctagctgcatcgtctaacgacgatgcagacaatgcagacgcctcggcgatcaatgcaggcaatccagagaaggaacttgattccgatgtgctggaacaagaactctccagcgaagaaccggaagaaacagcaaaaccagatcactctctccgaggcttcttccgcactgattactacccaaatcggtggcagaagatcctgtcgtttggcggacgtgtccgcatgagcacttccctgttgttgggtgcgctgctcttgctgtcactatttaaggtcatgactgtggaaccaagtgagaattggcaaaactccagtggatggctgtcaccaagcactgccacctcaactgcggtgaccacctccgaaacttccgcgccagcaagcacgccttcgatgacagtgcccactacggtggaggagaccccaacgatggaatctagcgtcgaaacgcagcaggaaacctcaacccctgcaaccgcaacgccccagcgagccgacaccatcgaaccgaccgaggaagccacgtcgcaggaggaaacgactgcatcgcagacgcagtctccagcagtggaagcaccaaccgcggtccaagaaacagttgcgccgacgtccaccccttag

SEQ ID NO: 8 - protein, 533 aa, Corynebacterium glutamicum
MILGVPIQYLLYSLWNWIVDTGFDVAIILVLAFLIPRIGRLAMRIIKQRVESAADADTTKNQLAFAGVGVYIAQIVAFFMLAVSAMQAFGFSLAGAAIPATIASAAIGLGAQSIVADFLAGFFILTEKQFGVGDWVRFEGNGIVVEGTVIEITMRATKIRTIAQETVIIPNSTAKVCINNSNNWSRAVVVIPIPMLGSENITDVIARSEAATRRALGQEKIAPEILGELDVHPATEVTPPTVVGMPWMVTMRFLVQVTAGNQWLVERAIRTEIINEFWEEYGSATTTSGTLIDSLHVEHEEPKTSLIDASPQALKEPKPEAAATVASLAASSNDDADNADASAINAGNPEKELDSDVLEQELSSEEPEETAKPDHSLRGFFRTDYYPNRWQKILSFGGRVRMSTSLLLGALLLLSLFKVMTVEPSENWQNSSGWLSPSTATSTAVTTSETSAPASTPSMTVPTTVEETPTMESSVETQQETSTPATATPQRADTIEPTEEATSQEETTASQTQSPAVEAPTAVQETVAPTSTP

SEQ ID NO: 9 - DNA, 3060 bp, Corynebacterium glutamicum
  source 1..3060: mol_type = genomic DNA
atgattttaggcgtacccattcaatatttgctctattcattgtggaattggattgtcgataccggttttgatgtagcaattatcctggtcttggcgtttttgattccacgtatcggccgactggccatgcgtattatcaagcagcgagtggagtctgcagccgatgcggacaccactaagaaccagctcgcgttcgctggcgttggcgtttatatcgcgcaaattgtggcgtttttcatgcttgccgtctccgcgatgcaggcttttggtttctctctcgcgggcgctgcgattccggcaaccattgcgtcagctgccattggtcttggtgcgcagtcgattgttgcggacttcttggccggatttttcatcctgacggaaaagcaattcggcgtgggtgactgggtgcgctttgagggcaacggcatcgttgttgaaggcaccgtcattgagatcaccatgcgcgcgaccaaaattcgcacgattgcacaagagaccgtgatcatcccgaactccacggcgaaagtgtgcatcaacaattctaataactggtcgcgtgcggttgtcgttattccgatccccatgttgggttctgaaaacatcacagatgtcatcgcgcgctctgaagctgcgactcgtcgcgcacttggccaggagaaaatcgcaccggaaatcctcggtgaactcgatgtgcacccagccacggaagtcacaccgccaacggtggtcggcatgccgtggatggtcaccatgcgtttcctcgtgcaagtcaccgccggcaatcaatggctggtcgaacgcgccatccgcacagaaatcatcaacgaattctgggaagaatacggcagcgcaaccactacatcgggaaccctcattgattccttacacgttgagcatgaagagccaaagacctcgcttatcgacgcctccccccaggctcttaaggaaccgaagccggaggctgcggcgacggttgcatcgctagctgcatcgtctaacgacgatgcagacaatgcagacgcctcggcgatcaatgcaggcaatccagagaaggaacttgattccgatgtgctggaacaagaactctccagcgaagaaccggaagaaacagcaaaaccagatcactctctccgaggcttcttccgcactgattactacccaaatcggtggcagaagatcctgtcgtttggcggacgtgtccgcatgagcacttccctgttgttgggtgcgctgctcttgctgtcactatttaaggggctcttcctgttttagagtgcattgatcttatggaccaactgccctgaatggataaggcaccgcagaatgtagtggttcaaattacggaaacctagagcaatcccacgcaaatgctccaaccgtccgttgatcgcttcgaccggaccgttggagacaccaacatcgaaatacgccaacacatcaccaagtcgtttaaacaaactacgacccaactgcgcgagttccttattcggccccttcaacacccgaagctgatcaataatggtccgcattttcttcttcgcttcacgcttattacccatctgataacaatcaataatcgcctgatacgcaagccacgcaagctttaacaccccgtagtctttgtcatacgcccacaactgctccaagctttcttgctgacgaggactcaaccacttgtgcgtggtcaacaaggtcttccggtttttatacaacggatcctggcttaaaccacgacgctggtatttctcccgctggaggcgttgccggcaggcggtgagcttgtcaccagcaagccgcacaacatggaatggatccatcacgcgacgagcagaaggaatgagttctttacttgctgtggcgtagccttggaacccatccatggacacgatccgtatctgattgcggaactgttcaccgcgggaaccaagccaggaccgtaaagcatcagcactacgacctgggacgacatctaataaccgggcaggacaccgtgagtcataccgatgcccggtcatatcgacaatcacggtgacaaacccatcaccatgcttagccctattatgtgaccacttatgctcatccaccccaatgacatacactccatcaagatggtgaggatcgttatagaccagctcacggcacatatcgagggctagttggcaggttaaatcccaccctagcccaagtgctttcgcggttgcgtgaacactcatccggtcaatagcaaggcgttgcaaaatccagcgggtgacccggtgggtgacctttttaccgtggtcagcgcagcttagttctgcttggaaatacttttgcttacatgtcgggttggtgcagcggtagcgaggtagacggataaacagtttggtgggaaacccgacgatgggtaaatcaatgagcatccggtgggtgtgatgacgaaacaccccaggttgggagcattctgggcaggtggaggtatagtcgagtgcgtctgcttcgatcagggtgtaatcacctgcatcggaagcgccggtgatggtgagtcctagttccgcagtgcggcagatggtgtcagcgatgatgttgccggtagacttcatgggtagagccttttgttggtgtttggttagcttagatacctaaaccttaaccctgacaaaaggctcgtttattttcgggtctacaccgctagcccaggttctgtgatgtaccccaaaaccggaagggccatttaaggtcatgactgtggaaccaagtgagaattggcaaaactccagtggatggctgtcaccaagcactgccacctcaactgcggtgaccacctccgaaacttccgcgccagcaagcacgccttcgatgacagtgcccactacggtggaggagaccccaacgatggaatctagcgtcgaaacgcagcaggaaacctcaacccctgcaaccgcaacgccccagcgagccgacaccatcgaaccgaccgaggaagccacgtcgcaggaggaaacgactgcatcgcagacgcagtctccagcagtggaagcaccaaccgcggtccaagaaacagttgcgccgacgtccacccct

SEQ ID NO: 10 - protein, 423 aa, Corynebacterium glutamicum
MILGVPIQYLLYSLWNWIVDTGFDVAIILVLAFLIPRIGRLAMRIIKQRVESAADADTTKNQLAFAGVGVYIAQIVAFFMLAVSAMQAFGFSLAGAAIPATIASAAIGLGAQSIVADFLAGFFILTEKQFGVGDWVRFEGNGIVVEGTVIEITMRATKIRTIAQETVIIPNSTAKVCINNSNNWSRAVVVIPIPMLGSENITDVIARSEAATRRALGQEKIAPEILGELDVHPATEVTPPTVVGMPWMVTMRFLVQVTAGNQWLVERAIRTEIINEFWEEYGSATTTSGTLIDSLHVEHEEPKTSLIDASPQALKEPKPEAAATVASLAASSNDDADNADASAINAGNPEKELDSDVLEQELSSEEPEETAKPDHSLRGFFRTDYYPNRWQKILSFGGRVRMSTSLLLGALLLLSLFKGLFLF